European Patent Application EP 4 180 799 A1, published May 17, 2023. Title: Methods and systems for detcting an analyte or classifying a sample. Applicant: Commonwealth Scientific and Industrial Research Organisation. Application EP 22191771.9, filed April 15, 2013. The sequence listing filed with the application follows.

SEQUENCE LISTING (46 sequences)

SEQ ID NO: 1 - DNA, 2670 bp, synthetic construct
  source 1..2670: mol_type = other DNA
atgtcgggagaattgtggattaccctagttgacacagcggacattgtcggcgtcaccctcaccttctgtgtcaacattgttcttctcggacttctgaaaacacgtggaaaaaacttgggcacttataaatatctcatggcgtttttctcagtattctcgattttttacgccatcatcgagttcatattacgacctataatgcatattgagaacaccactttctttttgatctcaaggaaaagattcaactactccaccaaacttggaaaaatcaactctgcgttttactgtgcttgttttgccaccagttttgttgtctcaggagttcactttgtttatcgatattttgcaacttgcaaaccgaatctacttcgtttgttcaacttgccaactcttctactttggccacttggttgcagtgtacccgtgacaatgtgggctagtgtctcatattttttgtatccagataccgagtacacggaagcggctgtcaccaatgtactaaataaccactataactggatcaaaaaggagaatgtatcgtacattgcatacgtctattaccaatacgaaaacggagtaaggcatatctacctcaaaaacttgcttggatgctttgttcattactttgtcatgtcgatgacgtttgttgtgatgttctactgcggatatgccacgtggaaaactatgaatgaacacaaggatgtatctgatagaactatggtgagcaagggcgaggagctgttcaccggggtggtgcccatcctggtcgagctggacggcgacgtaaacggccacaagttcagcgtgtccggcgagggcgagggcgatgccacctacggcaagctgaccctgaagttcatctgcaccaccggcaagctgcccgtgccctggcccaccctcgtgaccaccctgagctacggcgtgcagtgcttcagccgctaccccgaccacatgaagcagcacgacttcttcaagtccgccatgcccgaaggctacgtccaggagcgcaccatcttcttcaaggacgacggcaactacaagacccgcgccgaggtgaagttcgagggcgacaccctggtgaaccgcatcgagctgaagggcatcgacttcaaggaggacggcaacatcctggggcacaagctggagtacaactacaacagccacaacgtctatatcatggccgacaagcagaagaacggcatcaaggtgaacttcaagatccgccacaacatcgaggacggcagcgtgcagctcgccgaccactaccagcagaacacccccatcggcgacggccccgtgctgctgcccgacaaccactacctgagcacccagtccgccctgagcaaagaccccaacgagaagcgcgatcacatggtcctgctggagttcgtgaccgccgccgggatcactctcggcatggacgagctgtacaagcgagcgctacagaaacaacttttcaaagctttagttcttcagacactcatcccaactatcttcatgtacgccccaactggagtcatgttcatcgcaccgttttttgacgtgaatttgaatgcaaacgccaatttcattgtgttttgctcatttctgtacccgggactcgatccactcattctgattttgatcattcgtgatttccgaagaacaatattcaatttcttgtgtggaaagaaaaacagtgttgatgaatcccgctcgacaacaagagccaatttgtctcaagttccgacgatgaccagcaaggtgtacgaccccgagcagaggaagaggatgatcaccggcccccagtggtgggccaggtgcaagcagatgaacgtgctggacagcttcatcaactactacgacagcgagaagcacgccgagaacgccgtgatcttcctgcacggcaacgccgctagcagctacctgtggaggcacgtggtgccccacatcgagcccgtggccaggtgcatcatccccgatctgatcggcatgggcaagagcggcaagagcggcaacggcagctacaggctgctggaccactacaagtacctgaccgcctggttcgagctcctgaacctgcccaagaagatcatcttcgtgggccacgactggggcgccgccctggccttccactacagctacgagcaccaggacaagatcaaggccatcgtgcacgccgagagcgtggtggacgtgatcgagagctgggacgagtggccagacatcgaggaggacatcgccctgatcaagagcgaggagggcgagaagatggtgctggagaacaacttcttcgtggagaccgtgctgcccagcaagatcatgagaaagctggagcccgaggagttcgccgcctacctggagcccttcaaggagaagggcgaggtgagaagacccaccctgagctggcccagagagatccccctggtgaagggcggcaagcccgacgtggtgcagatcgtgagaaactacaacgcctacctgagagccagcgacgacctgcccaagatgttcatcgagagcgaccccggcttcttcagcaacgccatcgtggagggcgccaagaagttccccaacaccgagttcgtgaaggtgaagggcctgcacttcagccaggaggacgcccccgacgagatgggcaagtacatcaagagcttcgtggagagagtgctgaagaacgagcagtaa

SEQ ID NO: 2 - protein, 889 aa, synthetic construct
MSGELWITLVDTADIVGVTLTFCVNIVLLGLLKTRGKNLGTYKYLMAFFSVFSIFYAIIEFILRPIMHIENTTFFLISRKRFNYSTKLGKINSAFYCACFATSFVVSGVHFVYRYFATCKPNLLRLFNLPTLLLWPLGCSVPVTMWASVSYFLYPDTEYTEAAVTNVLNNHYNWIKKENVSYIAYVYYQYENGVRHIYLKNLLGCFVHYFVMSMTFVVMFYCGYATWKTMNEHKDVSDRTMVSKGEELFTGVVPILVELDGDVNGHKFSVSGEGEGDATYGKLTLKFICTTGKLPVPWPTLVTTLSYGVQCFSRYPDHMKQHDFFKSAMPEGYVQERTIFFKDDGNYKTRAEVKFEGDTLVNRIELKGIDFKEDGNILGHKLEYNYNSHNVYIMADKQKNGIKVNFKIRHNIEDGSVQLADHYQQNTPIGDGPVLLPDNHYLSTQSALSKDPNEKRDHMVLLEFVTAAGITLGMDELYKRALQKQLFKALVLQTLIPTIFMYAPTGVMFIAPFFDVNLNANANFIVFCSFLYPGLDPLILILIIRDFRRTIFNFLCGKKNSVDESRSTTRANLSQVPTMTSKVYDPEQRKRMITGPQWWARCKQMNVLDSFINYYDSEKHAENAVIFLHGNAASSYLWRHVVPHIEPVARCIIPDLIGMGKSGKSGNGSYRLLDHYKYLTAWFELLNLPKKIIFVGHDWGAALAFHYSYEHQDKIKAIVHAESVVDVIESWDEWPDIEEDIALIKSEEGEKMVLENNFFVETVLPSKIMRKLEPEEFAAYLEPFKEKGEVRRPTLSWPREIPLVKGGKPDVVQIVRNYNAYLRASDDLPKMFIESDPGFFSNAIVEGAKKFPNTEFVKVKGLHFSQEDAPDEMGKYIKSFVERVLKNEQ

SEQ ID NO: 3 - DNA, 2823 bp, synthetic construct
  source 1..2823: mol_type = other DNA
atggtgagcaagggcgaggagctgttcaccggggtggtgcccatcctggtcgagctggacggcgacgtaaacggccacaagttcagcgtgtccggcgagggcgagggcgatgccacctacggcaagctgaccctgaagttcatctgcaccaccggcaagctgcccgtgccctggcccaccctcgtgaccaccctgagctacggcgtgcagtgcttcagccgctaccccgaccacatgaagcagcacgacttcttcaagtccgccatgcccgaaggctacgtccaggagcgcaccatcttcttcaaggacgacggcaactacaagacccgcgccgaggtgaagttcgagggcgacaccctggtgaaccgcatcgagctgaagggcatcgacttcaaggaggacggcaacatcctggggcacaagctggagtacaactacaacagccacaacgtctatatcatggccgacaagcagaagaacggcatcaaggtgaacttcaagatccgccacaacatcgaggacggcagcgtgcagctcgccgaccactaccagcagaacacccccatcggcgacggccccgtgctgctgcccgacaaccactacctgagcacccagtccgccctgagcaaagaccccaacgagaagcgcgatcacatggtcctgctggagttcgtgaccgccgccgggatcactctcggcatggacgagctgtacaagctgcagggtggtaccggaggcggcatgaaaatcgaagaaggtaaactggtaatctggattaacggcgataaaggctataacggtctcgctgaagtcggtaagaaattcgagaaagataccggaattaaagtcaccgttgagcatccggataaactggaagagaaattcccacaggttgcggcaactggcgatggccctgacattatcttctgggcacacgaccgctttggtggctacgctcaatctggcctgttggctgaaatcaccccggacaaagcgttccaggacaagctgtatccgtttacctgggatgccgtacgttacaacggcaagctgattgcttacccgatcgctgttgaagcgttatcgctgatttataacaaagatctgctgccgaacccgccaaaaacctgggaagagatcccggcgctggataaagaactgaaagcgaaaggtaagagcgcgctgatgttcaacctgcaagaaccgtacttcacctggccgctgattgctgctgacgggggttatgcgttcaagtatgaaaacggcaagtacgacattaaagacgtgggcgtggataacgctggcgcgaaagcgggtctgaccttcctggttgacctgattaaaaacaaacacatgaatgcagacaccgattactccatcgcagaagctgcctttaataaaggcgaaacagcgatgaccatcaacggcccgtgggcatggtccaacatcgacaccagcaaagtgaattatggtgtaacggtactgccgaccttcaagggtcaaccatccaaaccgttcgttggcgtgctgagcgcaggtattaacgccgccagtccgaacaaagagctggcaaaagagttcctcgaaaactatctgctgactgatgaaggtctggaagcggttaataaagacaaaccgctgggtgccgtagcgctgaagtcttacgaggaagagttggtgaaagatccgcgtattgccgccactatggaaaacgcccagaaaggtgaaatcatgccgaacatcccgcagatgtccgctttctggtatgccgtgcgtactgcggtgatcaacgccgccagcggtcgtcagactgtcgatgaagccctgaaagacgcgcagactgccctgaaagacgcgcagactggcggcggtaccggtggattcgaaatggcttccaaggtgtacgaccccgagcaacgcaaacgcatgatcactgggcctcagtggtgggctcgctgcaagcaaatgaacgtgctggactccttcatcaactactatgattccgagaagcacgccgagaacgccgtgatttttctgcatggtaacgctgcctccagctacctgtggaggcacgtcgtgcctcacatcgagcccgtggctagatgcatcatccctgatctgatcggaatgggtaagtccggcaagagcgggaatggctcatatcgcctcctggatcactacaagtacctcaccgcttggttcgagctgctgaaccttccaaagaaaatcatctttgtgggccacgactggggggctgctctggcctttcactactcctacgagcaccaagacaagatcaaggccatcgtccatgctgagagtgtcgtggacgtgatcgagtcctgggacgagtggcctgacatcgaggaggatatcgccctgatcaagagcgaagagggcgagaaaatggtgcttgagaataacttcttcgtcgagaccgtgctcccaagcaagatcatgcggaaactggagcctgaggagttcgctgcctacctggagccattcaaggagaagggcgaggttagacggcctaccctctcctggcctcgcgagatccctctcgttaagggaggcaagcccgacgtcgtccagattgtccgcaactacaacgcctaccttcgggccagcgacgatctgcctaagatgttcatcgagtccgaccctgggttcttttccaacgctattgtcgagggagctaagaagttccctaacaccgagttcgtgaaggtgaagggcctccacttcagccaggaggacgctccagatgaaatgggtaagtacatcaagagcttcgtggagcgcgtgctgaagaacgagcagtaa

SEQ ID NO: 4 - protein, 940 aa, synthetic construct
MVSKGEELFTGVVPILVELDGDVNGHKFSVSGEGEGDATYGKLTLKFICTTGKLPVPWPTLVTTLSYGVQCFSRYPDHMKQHDFFKSAMPEGYVQERTIFFKDDGNYKTRAEVKFEGDTLVNRIELKGIDFKEDGNILGHKLEYNYNSHNVYIMADKQKNGIKVNFKIRHNIEDGSVQLADHYQQNTPIGDGPVLLPDNHYLSTQSALSKDPNEKRDHMVLLEFVTAAGITLGMDELYKLQGGTGGGMKIEEGKLVIWINGDKGYNGLAEVGKKFEKDTGIKVTVEHPDKLEEKFPQVAATGDGPDIIFWAHDRFGGYAQSGLLAEITPDKAFQDKLYPFTWDAVRYNGKLIAYPIAVEALSLIYNKDLLPNPPKTWEEIPALDKELKAKGKSALMFNLQEPYFTWPLIAADGGYAFKYENGKYDIKDVGVDNAGAKAGLTFLVDLIKNKHMNADTDYSIAEAAFNKGETAMTINGPWAWSNIDTSKVNYGVTVLPTFKGQPSKPFVGVLSAGINAASPNKELAKEFLENYLLTDEGLEAVNKDKPLGAVALKSYEEELVKDPRIAATMENAQKGEIMPNIPQMSAFWYAVRTAVINAASGRQTVDEALKDAQTALKDAQTGGGTGGFEMASKVYDPEQRKRMITGPQWWARCKQMNVLDSFINYYDSEKHAENAVIFLHGNAASSYLWRHVVPHIEPVARCIIPDLIGMGKSGKSGNGSYRLLDHYKYLTAWFELLNLPKKIIFVGHDWGAALAFHYSYEHQDKIKAIVHAESVVDVIESWDEWPDIEEDIALIKSEEGEKMVLENNFFVETVLPSKIMRKLEPEEFAAYLEPFKEKGEVRRPTLSWPREIPLVKGGKPDVVQIVRNYNAYLRASDDLPKMFIESDPGFFSNAIVEGAKKFPNTEFVKVKGLHFSQEDAPDEMGKYIKSFVERVLKNEQ

SEQ ID NO: 5 - DNA, 2823 bp, synthetic construct
  source 1..2823: mol_type = other DNA
atggtgagcaagggcgaggagctgttcaccggggtggtgcccatcctggtcgagctggacggcgacgtaaacggccacaagttcagcgtgtccggcgagggcgagggcgatgccacctacggcaagctgaccctgaagttcatctgcaccaccggcaagctgcccgtgccctggcccaccctcgtgaccaccctgagctacggcgtgcagtgcttcagccgctaccccgaccacatgaagcagcacgacttcttcaagtccgccatgcccgaaggctacgtccaggagcgcaccatcttcttcaaggacgacggcaactacaagacccgcgccgaggtgaagttcgagggcgacaccctggtgaaccgcatcgagctgaagggcatcgacttcaaggaggacggcaacatcctggggcacaagctggagtacaactacaacagccacaacgtctatatcatggccgacaagcagaagaacggcatcaaggtgaacttcaagatccgccacaacatcgaggacggcagcgtgcagctcgccgaccactaccagcagaacacccccatcggcgacggccccgtgctgctgcccgacaaccactacctgagcacccagtccgccctgagcaaagaccccaacgagaagcgcgatcacatggtcctgctggagttcgtgaccgccgccgggatcactctcggcatggacgagctgtacaagctgcagggtggtaccggaggcggcatgaaaatcgaagaaggtaaactggtaatctggattaacggcgataaaggctataacggtctcgctgaagtcggtaagaaattcgagaaagataccggaattaaagtcaccgttgagcatccggataaactggaagagaaattcccacaggttgcggcaactggcgatggccctgacattatcttctgggcacacgaccgctttggtggctacgctcaatctggcctgttggctgaaatcaccccggacaaagcgttccaggacaagctgtatccgtttacctgggatgccgtacgttacaacggcaagctgattgcttacccgatcgctgttgaagcgttatcgctgatttataacaaagatctgctgccgaacccgccaaaaacctgggaagagatcccggcgctggataaagaactgaaagcgaaaggtaagagcgcgctgatgttcaacctgcaagaaccgtacttcacctggccgctgattgctgctgacgggggttatgcgttcaagtatgaaaacggcaagtacgacattaaagacgtgggcgtggataacgctggcgcgaaagcgggtctgaccttcctggttgacctgattaaaaacaaacacatgaatgcagacaccgattactccatcgcagaagctgcctttaataaaggcgaaacagcgatgaccatcaacggcccgtgggcatggtccaacatcgacaccagcaaagtgaattatggtgtaacggtactgccgaccttcaagggtcaaccatccaaaccgttcgttggcgtgctgagcgcaggtattaacgccgccagtccgaacaaagagctggcaaaagagttcctcgaaaactatctgctgactgatgaaggtctggaagcggttaataaagacaaaccgctgggtgccgtagcgctgaagtcttacgaggaagagttggtgaaagatccgcgtattgccgccactatggaaaacgcccagaaaggtgaaatcatgccgaacatcccgcagatgtccgctttcgcgtatgccgtgcgtactgcggtgatcaacgccgccagcggtcgtcagactgtcgatgaagccctgaaagacgcgcagactgccctgaaagacgcgcagactggcggcggtaccggtggattcgaaatggcttccaaggtgtacgaccccgagcaacgcaaacgcatgatcactgggcctcagtggtgggctcgctgcaagcaaatgaacgtgctggactccttcatcaactactatgattccgagaagcacgccgagaacgccgtgatttttctgcatggtaacgctgcctccagctacctgtggaggcacgtcgtgcctcacatcgagcccgtggctagatgcatcatccctgatctgatcggaatgggtaagtccggcaagagcgggaatggctcatatcgcctcctggatcactacaagtacctcaccgcttggttcgagctgctgaaccttccaaagaaaatcatctttgtgggccacgactggggggctgctctggcctttcactactcctacgagcaccaagacaagatcaaggccatcgtccatgctgagagtgtcgtggacgtgatcgagtcctgggacgagtggcctgacatcgaggaggatatcgccctgatcaagagcgaagagggcgagaaaatggtgcttgagaataacttcttcgtcgagaccgtgctcccaagcaagatcatgcggaaactggagcctgaggagttcgctgcctacctggagccattcaaggagaagggcgaggttagacggcctaccctctcctggcctcgcgagatccctctcgttaagggaggcaagcccgacgtcgtccagattgtccgcaactacaacgcctaccttcgggccagcgacgatctgcctaagatgttcatcgagtccgaccctgggttcttttccaacgctattgtcgagggagctaagaagttccctaacaccgagttcgtgaaggtgaagggcctccacttcagccaggaggacgctccagatgaaatgggtaagtacatcaagagcttcgtggagcgcgtgctgaagaacgagcagtaa

SEQ ID NO: 6 - protein, 940 aa, synthetic construct
MVSKGEELFTGVVPILVELDGDVNGHKFSVSGEGEGDATYGKLTLKFICTTGKLPVPWPTLVTTLSYGVQCFSRYPDHMKQHDFFKSAMPEGYVQERTIFFKDDGNYKTRAEVKFEGDTLVNRIELKGIDFKEDGNILGHKLEYNYNSHNVYIMADKQKNGIKVNFKIRHNIEDGSVQLADHYQQNTPIGDGPVLLPDNHYLSTQSALSKDPNEKRDHMVLLEFVTAAGITLGMDELYKLQGGTGGGMKIEEGKLVIWINGDKGYNGLAEVGKKFEKDTGIKVTVEHPDKLEEKFPQVAATGDGPDIIFWAHDRFGGYAQSGLLAEITPDKAFQDKLYPFTWDAVRYNGKLIAYPIAVEALSLIYNKDLLPNPPKTWEEIPALDKELKAKGKSALMFNLQEPYFTWPLIAADGGYAFKYENGKYDIKDVGVDNAGAKAGLTFLVDLIKNKHMNADTDYSIAEAAFNKGETAMTINGPWAWSNIDTSKVNYGVTVLPTFKGQPSKPFVGVLSAGINAASPNKELAKEFLENYLLTDEGLEAVNKDKPLGAVALKSYEEELVKDPRIAATMENAQKGEIMPNIPQMSAFAYAVRTAVINAASGRQTVDEALKDAQTALKDAQTGGGTGGFEMASKVYDPEQRKRMITGPQWWARCKQMNVLDSFINYYDSEKHAENAVIFLHGNAASSYLWRHVVPHIEPVARCIIPDLIGMGKSGKSGNGSYRLLDHYKYLTAWFELLNLPKKIIFVGHDWGAALAFHYSYEHQDKIKAIVHAESVVDVIESWDEWPDIEEDIALIKSEEGEKMVLENNFFVETVLPSKIMRKLEPEEFAAYLEPFKEKGEVRRPTLSWPREIPLVKGGKPDVVQIVRNYNAYLRASDDLPKMFIESDPGFFSNAIVEGAKKFPNTEFVKVKGLHFSQEDAPDEMGKYIKSFVERVLKNEQ

SEQ ID NO: 7 - DNA, 33 bp, synthetic construct
  source 1..33: mol_type = other DNA
cacgactggggcgccgccctggccttccactac

SEQ ID NO: 8 - DNA, 33 bp, synthetic construct
  source 1..33: mol_type = other DNA
gtagtggaaggccagggcggcgccccagtcgtg

SEQ ID NO: 9 - DNA, 34 bp, synthetic construct
  source 1..34: mol_type = other DNA
cttcttcgtggagaccgtgctgcccagcaagatc

SEQ ID NO: 10 - DNA, 34 bp, synthetic construct
  source 1..34: mol_type = other DNA
gatcttgctgggcagcacggtctccacgaagaag

SEQ ID NO: 11 - DNA, 32 bp, synthetic construct
  source 1..32: mol_type = other DNA
cagatgtccgctttcgcgtatgccgtgcgtac

SEQ ID NO: 12 - DNA, 32 bp, synthetic construct
  source 1..32: mol_type = other DNA
gtacgcacggcatacgcgaaagcggacatctg

SEQ ID NO: 13 - protein, 896 aa, synthetic construct
MSGQLWLALVDAADMVGFTLTISINIILLGLIRTRGKTLGTYKYLMSFFSFFSIFYAIVESILRPIMHIENTTFFLISRKRFDYSTRLGKINSAFYCACFATSFVLSAVHFVYRYFAACKPNLLRLFNLPHLLLWPLMCSIPVTAWASVSYFLYPDTEYTEAAVTYVLKTHYEVIKKENVSYIAYVYYQYENGERHIYIKNLLGCFVHYFVMSMTFVVVFYCGFSTWWTIREHRGASDRTMVSKGEELFTGVVPILVELDGDVNGHKFSVSGEGEGDATYGKLTLKFICTTGKLPVPWPTLVTTLTYGVQCFSRYPDHMKQHDFFKSAMPEGYVQERTIFFKDDGNYKTRAEVKFEGDTLVNRIELKGIDFKEDGNILGHKLEYNYNSHNVYIMADKQKNGIKVNFKIRHNIEDGSVQLADHYQQNTPIGDGPVLLPDNHYLSTQSALSKDPNEKRDHMVLLEFVTAAGITLGMDELYKRHLHRQLFKALVFQTLVPSIFMYIPTGVMFIAPFFDINLNANANFIVFCSFLYPGLDPLILIFIIREFRVTILNIIRGNERGNAVGEAYSTSRIKSSQPAAVNLSGMTSKVYDPEQRKRMITGPQWWARCKQMNVLDSFINYYDSEKHAENAVIFLHGNAASSYLWRHVVPHIEPVARCIIPDLIGMGKSGKSGNGSYRLLDHYKYLTAWFELLNLPKKIIFVGHDWGACLAFHYSYEHQDKIKAIVHAESVVDVIESWDEWPDIEEDIALIKSEEGEKMVLENNFFVETMLPSKIMRKLEPEEFAAYLEPFKEKGEVRRPTLSWPREIPLVKGGKPDVVQIVRNYNAYLRASDDLPKMFIESDPGFFSNAIVEGAKKFPNTEFVKVKGLHFSQEDAPDEMGKYIKSFVERVLKNEQ

SEQ ID NO: 14 - protein, 897 aa, synthetic construct
MSDRHWLDITTYSDHIGFTISTIANFVLILLLVFRPTKSYGSYKYLMITFCVFSLFYTSIETFLRPLIHIYDNTIFVIQRKRFQYSEGTARAISSTYCGCYAMSFTLFAVHFVYRYYAACKPDNLRYFQGCYFVAWVFGAMAVAASWGFAAFILYPETERTRTALIHVIQTSYELDPEWVGNVPYSYWRTENGVEYLNPRNVIGIFQHGVIMILSFGTVFYCGFNTYKTLNGSLGVSEKTSGMVSKGEELFTGVVPILVELDGDVNGHKFSVSGEGEGDATYGKLTLKFICTTGKLPVPWPTLVTTLSYGVQCFSRYPDHMKQHDFFKSAMPEGYVQERTIFFKDDGNYKTRAEVKFEGDTLVNRIELKGIDFKEDGNILGHKLEYNYNSHNVYIMADKQKNGIKVNFKIRHNIEDGSVQLADHYQQNTPIGDGPVLLPDNHYLSTQSALSKDPNEKRDHMVLLEFVTAAGITLGMDELYKVDKEMHTQLFKALVLQTIIPTTLMYIPTTMLFVTPFVGLNIGCYGNITTATVHLYPGIDPVVLIFIIRDFRQTILRPFRCFYRSNSVENTATIRQYQQSSSKGSRMTSKVYDPEQRKRMITGPQWWARCKQMNVLDSFINYYDSEKHAENAVIFLHGNAASSYLWRHVVPHIEPVARCIIPDLIGMGKSGKSGNGSYRLLDHYKYLTAWFELLNLPKKIIFVGHDWGACLAFHYSYEHQDKIKAIVHAESVVDVIESWDEWPDIEEDIALIKSEEGEKMVLENNFFVETMLPSKIMRKLEPEEFAAYLEPFKEKGEVRRPTLSWPREIPLVKGGKPDVVQIVRNYNAYLRASDDLPKMFIESDPGFFSNAIVEGAKKFPNTEFVKVKGLHFSQEDAPDEMGKYIKSFVERVLKNEQ

SEQ ID NO: 15 - protein, 904 aa, synthetic construct
MSDIYWIQITEVCSFVGFMLSVLGNSTLLVLLSGKSIDGIGTYRYLMITFCVFSLLFTILEDFIRPLMHHYNNTIIVLQRKRFQFSDSTARILTVSYCGCFAMCFVMFAVHFIYRYLVACHPTKLHYFRPKNFIFWLSGMLFIAGSWVAIAYVFFQEDLETRTDLVFILSTCYNLTPDDVGHVPYAFYKTQGNTRVIRWDNMIGVIHHMIVMTISISAVFYFGIKTYTRIMSFKGKSQKTSGMVSKGEELFTGVVPILVELDGDVNGHKFSVSGEGEGDATYGKLTLKFICTTGKLPVPWPTLVTTLSYGVQCFSRYPDHMKQHDFFKSAMPEGYVQERTIFFKDDGNYKTRAEVKFEGDTLVNRIELKGIDFKEDGNILGHKLEYNYNSHNVYIMADKQKNGIKVNFKIRHNIEDGSVQLADHYQQNTPIGDGPVLLPDNHYLSTQSALSKDPNEKRDHMVLLEFVTAAGITLGMDELYKVDKDLQNQFFTALVAQTVVPLIFMFIPNMVLTTAALIDGTFGSWANITVVMNHLYPAADPFVILFIIKGFRNSIRNVIYRCTKTKKASVSSVVRGIEAQSKKQSFSRVDISRMTSKVYDPEQRKRMITGPQWWARCKQMNVLDSFINYYDSEKHAENAVIFLHGNAASSYLWRHVVPHIEPVARCIIPDLIGMGKSGKSGNGSYRLLDHYKYLTAWFELLNLPKKIIFVGHDWGACLAFHYSYEHQDKIKAIVHAESVVDVIESWDEWPDIEEDIALIKSEEGEKMVLENNFFVETMLPSKIMRKLEPEEFAAYLEPFKEKGEVRRPTLSWPREIPLVKGGKPDVVQIVRNYNAYLRASDDLPKMFIESDPGFFSNAIVEGAKKFPNTEFVKVKGLHFSQEDAPDEMGKYIKSFVERVLKNEQ

SEQ ID NO: 16 - protein, 890 aa, synthetic construct
MTDQHWVIITDIAGPIGFSMSIFSNSILLFLIFSHSSPIKGPYKRMLIVFCIFTVFYSFVEVMLQPLIHIYDDTLFLIHRKRIDLPKWLTRLVPTTYCWCYAMSFSLFALQFLYRYVAVCKPQYVDLFVGCHFYAWVVLILSLATSWGLTAAFMFPQTDRTTEIFLHIIYSSYDLEPYWTDYVAYKYFDTDENNVRWVNVLSFFGVLQHGIVITLSFGTLYYCGINTYLKIKKHTGTSNRTSGMVSKGEELFTGVVPILVELDGDVNGHKFSVSGEGEGDATYGKLTLKFICTTGKLPVPWPTLVTTLSYGVQCFSRYPDHMKQHDFFKSAMPEGYVQERTIFFKDDGNYKTRAEVKFEGDTLVNRIELKGIDFKEDGNILGHKLEYNYNSHNVYIMADKQKNGIKVNFKIRHNIEDGSVQLADHYQQNTPIGDGPVLLPDNHYLSTQSALSKDPNEKRDHMVLLEFVTAAGITLGMDELYKVDRCIQLQLFRALVAQTILPMFMMYIPVGFMFACPYFDLQLGAYTNYQTVMAQLYPGIDPFVMLFLIDSYRITIFGWLCPRFVYVKPMHSTYTLTSRMTSKVYDPEQRKRMITGPQWWARCKQMNVLDSFINYYDSEKHAENAVIFLHGNAASSYLWRHVVPHIEPVARCIIPDLIGMGKSGKSGNGSYRLLDHYKYLTAWFELLNLPKKIIFVGHDWGACLAFHYSYEHQDKIKAIVHAESVVDVIESWDEWPDIEEDIALIKSEEGEKMVLENNFFVETMLPSKIMRKLEPEEFAAYLEPFKEKGEVRRPTLSWPREIPLVKGGKPDVVQIVRNYNAYLRASDDLPKMFIESDPGFFSNAIVEGAKKFPNTEFVKVKGLHFSQEDAPDEMGKYIKSFVERVLKNEQ

SEQ ID NO: 17 - protein, 906 aa, synthetic construct
MTDRRWVAITDIAGPIGFTMSIFSNSVLLSLIFSSSSPIKGAYKNMLIVLCIFTMFYSFVEIMLQPLIHIYDDTLFLIHRKRFDLSKGITRLIPTTYCWCYAMSFSLFALQFLYRYVAVCKPHLVVFFTGCYFYYWLALILSLATSWGLTAAFMFPQTNRTTESFNYVIKTSYDLDPYWTDYVAYKYFDTDENHVRWVNVLSLFGVLQHGLVITLSFGTLFYCGIKTYLSITEHVGMSSKTSGMVSKGEELFTGVVPILVELDGDVNGHKFSVSGEGEGDATYGKLTLKFICTTGKLPVPWPTLVTTLSYGVQCFSRYPDHMKQHDFFKSAMPEGYVQERTIFFKDDGNYKTRAEVKFEGDTLVNRIELKGIDFKEDGNILGHKLEYNYNSHNVYIMADKQKNGIKVNFKIRHNIEDGSVQLADHYQQNTPIGDGPVLLPDNHYLSTQSALSKDPNEKRDHMVLLEFVTAAGITLGMDELYKVDRSLQLQLFRALVAQTCLPMLMMYMPIGFMFSCPYFDLQLGAVTNYQTVMAQLYPGIDPFMLLFLINAYRKTVLSLICPNFIQKKYVQTATTRDGTDASATMNSVKSTQLSRMTSKVYDPEQRKRMITGPQWWARCKQMNVLDSFINYYDSEKHAENAVIFLHGNAASSYLWRHVVPHIEPVARCIIPDLIGMGKSGKSGNGSYRLLDHYKYLTAWFELLNLPKKIIFVGHDWGACLAFHYSYEHQDKIKAIVHAESVVDVIESWDEWPDIEEDIALIKSEEGEKMVLENNFFVETMLPSKIMRKLEPEEFAAYLEPFKEKGEVRRPTLSWPREIPLVKGGKPDVVQIVRNYNAYLRASDDLPKMFIESDPGFFSNAIVEGAKKFPNTEFVKVKGLHFSQEDAPDEMGKYIKSFVERVLKNEQ

SEQ ID NO: 18 - protein, 901 aa, synthetic construct
MSDIYWIQITEVCSFVGFMLSVLGNSTLLVLLSGKSIDGIGTYRYLMITFCVFSLLFTILEDFIRPLMHHYNNTIIVLQRKRFQFSDSTARILTVSYCGCFAMCFVMFAVHFIYRYLVACHPTKLHYFRPKNFIFWLSGMLFIAGSWVAIAYVFFQEDLETRTDLVFILSTCYNLTPDDVGHVPYAFYKTQGNTRVIRWDNMIGVIHHMIVMTISISAVFYFGIKTYTRIMSFKGKSQKTSGMVSKGEELFTGVVPILVELDGDVNGHKFSVSGEGEGDATYGKLTLKFICTTGKLPVPWPTLVTTLSYGVQCFSRYPDHMKQHDFFKSAMPEGYVQERTIFFKDDGNYKTRAEVKFEGDTLVNRIELKGIDFKEDGNILGHKLEYNYNSHNVYIMADKQKNGIKVNFKIRHNIEDGSVQLADHYQQNTPIGDGPVLLPDNHYLSTQSALSKDPNEKRDHMVLLEFVTAAGITLGMDELYKVDKEMHTQLFKALVLQTIIPTTLMYIPTTMLFVTPFVGLNIGCYGNITTATVHLYPGIDPVVLIFIIRDFRQTILRPFRCFYRSNSVENTATIRQYQQSSSKGSREFGTMASKVYDPEQRKRMITGPQWWARCKQMNVLDSFINYYDSEKHAENAVIFLHGNAASSYLWRHVVPHIEPVARCIIPDLIGMGKSGKSGNGSYRLLDHYKYLTAWFELLNLPKKIIFVGHDWGAALAFHYSYEHQDKIKAIVHAESVVDVIESWDEWPDIEEDIALIKSEEGEKMVLENNFFVETVLPSKIMRKLEPEEFAAYLEPFKEKGEVRRPTLSWPREIPLVKGGKPDVVQIVRNYNAYLRASDDLPKMFIESDPGFFSNAIVEGAKKFPNTEFVKVKGLHFSQEDAPDEMGKYIKSFVERVLKNEQ

SEQ ID NO: 19 - DNA, 2694 bp, synthetic construct
  source 1..2694: mol_type = other DNA
atgggttctggtcaattatggttggctttagttgatgctgcagatatggttggttttactttgacaatctcaattaatatcattttgttaggtttgattagaactagaggtaaaaccttgggtacttacaagtacttgatgtctttcttttctttcttttctattttctatgcaatcgttgaatctatcttgagaccaatcatgcatatcgaaaacactacatttttcttaatctccagaaagagattcgattacagtactagattgggtaaaattaattcagctttctactgtgcttgtttcgcaacatccttcgttttgagtgcagttcatttcgtttacagatacttcgctgcttgtaagcctaatttgttgagattgtttaacttacctcatttgttattgtggccattgatgtgttcaattcctgttactgcttgggcatctgtttcatactttttgtacccagatacagaatataccgaagctgcagttacctatgttttgaagactcattacgaagttattaaaaaggaaaacgtttcttacattgcttacgtttactaccaatacgaaaacggtgaaagacatatctatattaaaaacttattgggttgtttcgttcattacttcgttatgtctatgacattcgttgttgttttctattgtggtttctcaacttggtggacaattagagaacatagaggtgcttccgatagaacaatggttagtaagggtgaagaattattcaccggtgttgttccaattttggttgaattagatggtgacgttaatggtcataaattttccgttagtggtgaaggtgaaggtgacgcaacatacggtaaattgaccttgaagtttatttgtaccactggtaaattgccagttccttggccaaccttggttacaaccttaacttatggtgttcaatgtttttccagataccctgatcatatgaagcaacatgatttctttaagagtgctatgccagaaggttacgttcaagaaagaacaattttctttaaggatgatggtaactacaagactagagcagaggttaagttcgaaggtgacacattggttaacagaatcgaattgaagggtatcgatttcaaggaagatggtaacatcttgggtcataagttggaatacaattacaactcccataacgtttacatcatggctgataagcaaaagaatggtattaaagttaacttcaagatcagacataacatcgaagatggttcagttcaattggcagatcattaccaacaaaacacccctattggtgacggtcctgttttgttgccagataaccattacttatcaactcaatccgctttgagtaaggatccaaacgaaaagagagatcatatggttttgttggaattcgttactgctgcaggtatcacattgggtatggatgaattgtacaagagacatttgcatagacaattgtttaaagctttggttttccaaaccttggttccatcaatttttatgtacatccctactggtgttatgttcatcgcaccatttttcgatatcaatttgaacgctaacgcaaacttcatcgttttctgttcatttttgtatcctggtttggatccattgatcttgattttcattatcagagaattcagagttacaattttaaacattattcgtggtaatgaacgtggtaacgctgttggtgaagcatactctacctcaagaattaaatcttcacaaccagctgcagttaatttgtctggtatgacatcaaaggtttacgatcctgaacaaagaaaaagaatgattaccggtccacaatggtgggctcgttgtaagcaaatgaacgttttggattctttcattaactactacgattcagaaaagcatgctgaaaacgctgttattttcttgcatggtaacgctgcatccagttatttgtggagacatgttgttcctcatattgaaccagttgctagatgtatcatccctgatttgatcggtatgggtaaatctggtaaatctggtaacggttcttacagattgttggatcattacaagtacttaactgcatggttcgaattgttgaatttgccaaagaaaattatcttcgttggtcatgattggggtgcttgtttggcatttcattactcttacgaacatcaagataaaattaaggctatcgttcatgcagaatccgttgttgatgttattgaaagttgggatgaatggccagatatcgaagaagatatcgctttaattaagtccgaagaaggtgaaaagatggttttggaaaacaactttttcgttgaaactatgttgcctagtaagatcatgagaaagttggaacctgaagaatttgctgcatatttggaaccattcaaagaaaagggtgaagttagaagacctacattatcttggcctagagaaattccattggttaaaggtggtaaaccagatgttgttcaaatcgttagaaactacaacgcttacttaagagcatctgatgatttgccaaagatgttcatcgaatctgatcctggtttcttttctaatgctattgttgaaggtgctaagaaattccctaacacagaattcgttaaggttaagggtttgcatttctctcaagaagatgctccagatgaaatgggtaaatacatcaagtcatttgttgaaagagttttgaaaaatgaacaataa

SEQ ID NO: 20 - DNA, 2694 bp, synthetic construct
  source 1..2694: mol_type = other DNA
atgtctgaccgtcattggctcgacatcaccacctactcagaccacattgggtttacgatttccaccatcgccaatttcgttctgatccttctgctagtcttccgaccgaccaaatcatacggttcatacaagtacctgatgatcacattctgcgtgttcagcctcttttacacctccattgaaacttttttgagacctctcatccatatctacgacaatacgatcttcgtgattcagcgcaagagattccagtactccgagggtaccgctagagccatttcatcgacctactgcggctgctacgccatgagcttcaccctgttcgccgtccactttgtctaccgttactatgcggcttgcaaacccgacaacctccgttacttccaaggatgctactttgtcgcatgggtattcggagcaatggcggtggcggcgagctgggggttcgcagcgtttattctgtacccggagaccgagaggaccaggacggcgttgatacacgtcatacaaacatcctatgagctggatcccgagtgggtgggaaatgttccatatagctattggcgcacagaaaacggagtggaatacctgaatcctcgcaacgtcatcgggatctttcaacacggcgtcatcatgatcctctccttcggaacagtcttctactgcggattcaacacttataagactttgaacggaagtctgggggtgtctgaaaaaacatccggaatggtgagcaagggcgaggagctgttcaccggggtggtgcccatcctggtcgagctggacggcgacgtaaacggccacaagttcagcgtgtccggcgagggcgagggcgatgccacctacggcaagctgaccctgaagttcatctgcaccaccggcaagctgcccgtgccctggcccaccctcgtgaccaccctgagctacggcgtgcagtgcttcagccgctaccccgaccacatgaagcagcacgacttcttcaagtccgccatgcccgaaggctacgtccaggagcgcaccatcttcttcaaggacgacggcaactacaagacccgcgccgaggtgaagttcgagggcgacaccctggtgaaccgcatcgagctgaagggcatcgacttcaaggaggacggcaacatcctggggcacaagctggagtacaactacaacagccacaacgtctatatcatggccgacaagcagaagaacggcatcaaggtgaacttcaagatccgccacaacatcgaggacggcagcgtgcagctcgccgaccactaccagcagaacacccccatcggcgacggccccgtgctgctgcccgacaaccactacctgagcacccagtccgccctgagcaaagaccccaacgagaagcgcgatcacatggtcctgctggagttcgtgaccgccgccgggatcactctcggcatggacgagctgtacaaggtcgacaaagaaatgcacacccaattgttcaaggccttggttctacagactatcatccctactacactaatgtacatcccgacaaccatgctctttgtcaccccattcgttggactcaacatcggctgttacggcaacatcactactgccaccgtccatttgtatcctggaattgacccagtcgttttgatctttataatccgagacttccggcaaacgattttaagaccattcagatgcttctaccgttcaaatagtgtcgaaaacactgccaccataaggcaataccagcagagcagctccaaaggatctagaatgaccagcaaggtgtacgaccccgagcagaggaagaggatgatcaccggcccccagtggtgggccaggtgcaagcagatgaacgtgctggacagcttcatcaactactacgacagcgagaagcacgccgagaacgccgtgatcttcctgcacggcaacgccgctagcagctacctgtggaggcacgtggtgccccacatcgagcccgtggccaggtgcatcatccccgatctgatcggcatgggcaagagcggcaagagcggcaacggcagctacaggctgctggaccactacaagtacctgaccgcctggttcgagctcctgaacctgcccaagaagatcatcttcgtgggccacgactggggcgcctgcctggccttccactacagctacgagcaccaggacaagatcaaggccatcgtgcacgccgagagcgtggtggacgtgatcgagagctgggacgagtggccagacatcgaggaggacatcgccctgatcaagagcgaggagggcgagaagatggtgctggagaacaacttcttcgtggagaccatgctgcccagcaagatcatgagaaagctggagcccgaggagttcgccgcctacctggagcccttcaaggagaagggcgaggtgagaagacccaccctgagctggcccagagagatccccctggtgaagggcggcaagcccgacgtggtgcagatcgtgagaaactacaacgcctacctgagagccagcgacgacctgcccaagatgttcatcgagagcgaccccggcttcttcagcaacgccatcgtggagggcgccaagaagttccccaacaccgagttcgtgaaggtgaagggcctgcacttcagccaggaggacgcccccgacgagatgggcaagtacatcaagagcttcgtggagagagtgctgaagaacgagcagtaa

SEQ ID NO: 21 - DNA, 2715 bp, synthetic construct
  source 1..2715: mol_type = other DNA
atgtccgatatatactggatacaaattactgaagtttgctccttcgtcggatttatgctctcagttctagggaacagtacacttttagtactgctcagtggaaaatccatagatggaattggcacctatcggtacttgatgatcactttctgcgttttcagtttattatttacgatattagaggattttatcagaccgctgatgcatcactataacaataccataattgttttacaacgcaagcggtttcagttttctgattcaacggctagaatcttgacagtctcttactgcggctgtttcgcgatgtgcttcgtgatgttcgccgttcatttcatctatcgatatctagttgcttgtcacccgacaaaattgcactattttcgacccaaaaatttcattttctggctgtccggcatgttattcatagcaggaagctgggttgcaattgcatatgtcttttttcaagaagacctagaaaccaggacggatttggtatttattttgtcaacttgttataatttaacgccagatgatgtcggacatgtaccgtatgctttttacaaaactcaaggaaatacacgagtaattcgatgggataacatgattggagtaattcatcatatgatagttatgacaatctctataagtgccgttttctactttggcattaaaacctacactcgaataatgagtttcaagggaaaatcccagaaaacctccggaatggtgagcaagggcgaggagctgttcaccggggtggtgcccatcctggtcgagctggacggcgacgtaaacggccacaagttcagcgtgtccggcgagggcgagggcgatgccacctacggcaagctgaccctgaagttcatctgcaccaccggcaagctgcccgtgccctggcccaccctcgtgaccaccctgagctacggcgtgcagtgcttcagccgctaccccgaccacatgaagcagcacgacttcttcaagtccgccatgcccgaaggctacgtccaggagcgcaccatcttcttcaaggacgacggcaactacaagacccgcgccgaggtgaagttcgagggcgacaccctggtgaaccgcatcgagctgaagggcatcgacttcaaggaggacggcaacatcctggggcacaagctggagtacaactacaacagccacaacgtctatatcatggccgacaagcagaagaacggcatcaaggtgaacttcaagatccgccacaacatcgaggacggcagcgtgcagctcgccgaccactaccagcagaacacccccatcggcgacggccccgtgctgctgcccgacaaccactacctgagcacccagtccgccctgagcaaagaccccaacgagaagcgcgatcacatggtcctgctggagttcgtgaccgccgccgggatcactctcggcatggacgagctgtacaaggtcgacaaggatctccagaatcaatttttcactgctctagttgctcaaaccgtagtccctctgattttcatgtttatcccaaatatggtgctcactacggcagcccttatagatggcacatttggctcatgggccaatattactgtagttatgaatcatttgtatccggctgccgatccattcgttatactgttcattattaaggggttccggaatagtattagaaatgttatatatcgctgcacaaaaacgaaaaaagcatcggttagctcagtggtccgtggtattgaggctcaaagcaagaaacaatctttttctcgagttgatatttctagaatgaccagcaaggtgtacgaccccgagcagaggaagaggatgatcaccggcccccagtggtgggccaggtgcaagcagatgaacgtgctggacagcttcatcaactactacgacagcgagaagcacgccgagaacgccgtgatcttcctgcacggcaacgccgctagcagctacctgtggaggcacgtggtgccccacatcgagcccgtggccaggtgcatcatccccgatctgatcggcatgggcaagagcggcaagagcggcaacggcagctacaggctgctggaccactacaagtacctgaccgcctggttcgagctcctgaacctgcccaagaagatcatcttcgtgggccacgactggggcgcctgcctggccttccactacagctacgagcaccaggacaagatcaaggccatcgtgcacgccgagagcgtggtggacgtgatcgagagctgggacgagtggccagacatcgaggaggacatcgccctgatcaagagcgaggagggcgagaagatggtgctggagaacaacttcttcgtggagaccatgctgcccagcaagatcatgagaaagctggagcccgaggagttcgccgcctacctggagcccttcaaggagaagggcgaggtgagaagacccaccctgagctggcccagagagatccccctggtgaagggcggcaagcccgacgtggtgcagatcgtgagaaactacaacgcctacctgagagccagcgacgacctgcccaagatgttcatcgagagcgaccccggcttcttcagcaacgccatcgtggagggcgccaagaagttccccaacaccgagttcgtgaaggtgaagggcctgcacttcagccaggaggacgcccccgacgagatgggcaagtacatcaagagcttcgtggagagagtgctgaagaacgagcagtaa

SEQ ID NO: 22 - DNA, 2673 bp, synthetic construct
  source 1..2673: mol_type = other DNA
atgactgatcaacactgggttattatcacagatattgctggtccaatcggattttcaatgtccattttttcaaactctattcttttgtttttgatattttcacattcatctccaataaaaggtccatacaaacgaatgctcatagtattttgcatatttaccgtattctactcatttgtcgaagtcatgcttcagccactaatccatatttacgacgacactttatttttgattcatcgaaagagaatagacttgccaaaatggttaacacgtttggttcctactacctattgttggtgttacgcaatgagtttttccttgtttgcattacaatttttatatagatatgtggcagtatgcaaaccgcaatatgttgatctttttgtcggatgtcacttttatgcttgggtagttttgatcttatcactagccacgagctggggactcactgcagctttcatgttcccacaaaccgaccgaacaactgaaatttttttgcacataatttatagttcatatgacttggagccttattggacagattatgttgcttataaatactttgatactgatgagaataatgtgagatgggtcaatgttcttagttttttcggtgtccttcagcacgggattgtaattactctaagttttggcaccctttattattgtggcatcaacacgtatctcaaaataaaaaaacacactggaacatcaaacagaacttccggaatggtgagcaagggcgaggagctgttcaccggggtggtgcccatcctggtcgagctggacggcgacgtaaacggccacaagttcagcgtgtccggcgagggcgagggcgatgccacctacggcaagctgaccctgaagttcatctgcaccaccggcaagctgcccgtgccctggcccaccctcgtgaccaccctgagctacggcgtgcagtgcttcagccgctaccccgaccacatgaagcagcacgacttcttcaagtccgccatgcccgaaggctacgtccaggagcgcaccatcttcttcaaggacgacggcaactacaagacccgcgccgaggtgaagttcgagggcgacaccctggtgaaccgcatcgagctgaagggcatcgacttcaaggaggacggcaacatcctggggcacaagctggagtacaactacaacagccacaacgtctatatcatggccgacaagcagaagaacggcatcaaggtgaacttcaagatccgccacaacatcgaggacggcagcgtgcagctcgccgaccactaccagcagaacacccccatcggcgacggccccgtgctgctgcccgacaaccactacctgagcacccagtccgccctgagcaaagaccccaacgagaagcgcgatcacatggtcctgctggagttcgtgaccgccgccgggatcactctcggcatggacgagctgtacaaggtcgaccgatgtattcaactacaacttttcagagctctggttgcacagacaattttaccaatgttcatgatgtatattcccgttggtttcatgtttgcatgtccatattttgacttgcaattaggtgcatacaccaattatcaaacagtcatggcacaactttatccgggaatcgacccatttgtgatgctgtttttgatagattcttatagaataacaatatttggatggttatgtccaagatttgtttatgtaaagccgatgcattccacatacaccctaacttctagaatgaccagcaaggtgtacgaccccgagcagaggaagaggatgatcaccggcccccagtggtgggccaggtgcaagcagatgaacgtgctggacagcttcatcaactactacgacagcgagaagcacgccgagaacgccgtgatcttcctgcacggcaacgccgctagcagctacctgtggaggcacgtggtgccccacatcgagcccgtggccaggtgcatcatccccgatctgatcggcatgggcaagagcggcaagagcggcaacggcagctacaggctgctggaccactacaagtacctgaccgcctggttcgagctcctgaacctgcccaagaagatcatcttcgtgggccacgactggggcgcctgcctggccttccactacagctacgagcaccaggacaagatcaaggccatcgtgcacgccgagagcgtggtggacgtgatcgagagctgggacgagtggccagacatcgaggaggacatcgccctgatcaagagcgaggagggcgagaagatggtgctggagaacaacttcttcgtggagaccatgctgcccagcaagatcatgagaaagctggagcccgaggagttcgccgcctacctggagcccttcaaggagaagggcgaggtgagaagacccaccctgagctggcccagagagatccccctggtgaagggcggcaagcccgacgtggtgcagatcgtgagaaactacaacgcctacctgagagccagcgacgacctgcccaagatgttcatcgagagcgaccccggcttcttcagcaacgccatcgtggagggcgccaagaagttccccaacaccgagttcgtgaaggtgaagggcctgcacttcagccaggaggacgcccccgacgagatgggcaagtacatcaagagcttcgtggagagagtgctgaagaacgagcagtaa

SEQ ID NO: 23 - DNA, 2721 bp, synthetic construct
  source 1..2721: mol_type = other DNA
atgaccgatcgtcgctgggtcgctattacggacattgccggaccgattgggttcacaatgtcaattttttcgaactcggtgctgttatcgttgatattctcaagcagctctccaattaaaggagcttacaaaaatatgttgatagtgttgtgtatattcactatgttctactcttttgttgaaataatgcttcaaccgttgattcatatttatgatgacacgctgttcttgatccaccggaaaagatttgacctgtctaaaggaattacacgtttgatacctacaacatattgttggtgttatgcaatgagtttctcattattcgccctccagtttttgtacagatatgtggcagtttgcaaacctcacttagttgttttttttactggatgctatttctattattggttggcactcatcttatcacttgctacaagttgggggcttactgcagcttttatgttcccgcaaaccaatcgaacaactgaaagcttcaactacgtaataaaaacttcttatgacttagatccttattggacggattatgttgcctataaatattttgacaccgatgagaatcatgtgagatgggtgaatgttcttagtttatttggagtcttgcagcacggattagtaattacgttgagttttggaaccttattctactgtggaattaaaacttatctcagcattactgaacatgttggaatgtccagcaagacctccggaatggtgagcaagggcgaggagctgttcaccggggtggtgcccatcctggtcgagctggacggcgacgtaaacggccacaagttcagcgtgtccggcgagggcgagggcgatgccacctacggcaagctgaccctgaagttcatctgcaccaccggcaagctgcccgtgccctggcccaccctcgtgaccaccctgagctacggcgtgcagtgcttcagccgctaccccgaccacatgaagcagcacgacttcttcaagtccgccatgcccgaaggctacgtccaggagcgcaccatcttcttcaaggacgacggcaactacaagacccgcgccgaggtgaagttcgagggcgacaccctggtgaaccgcatcgagctgaagggcatcgacttcaaggaggacggcaacatcctggggcacaagctggagtacaactacaacagccacaacgtctatatcatggccgacaagcagaagaacggcatcaaggtgaacttcaagatccgccacaacatcgaggacggcagcgtgcagctcgccgaccactaccagcagaacacccccatcggcgacggccccgtgctgctgcccgacaaccactacctgagcacccagtccgccctgagcaaagaccccaacgagaagcgcgatcacatggtcctgctggagttcgtgaccgccgccgggatcactctcggcatggacgagctgtacaaggtcgaccgaagtcttcaacttcaactattccgtgctttagttgctcagacatgtcttccaatgctcatgatgtacatgccaataggattcatgttttcttgcccttactttgatttgcaacttggagcagtcacaaactatcaaaccgtcatggcacagttatacccaggaatcgacccatttatgttgctatttcttattaacgcctacagaaagacagtgttaagcttgatctgtcctaattttatccagaaaaaatatgttcaaacggcaactactcgtgatggcacagatgcctcggcaacaatgaattctgttaaatctacacagttatctagaatgaccagcaaggtgtacgaccccgagcagaggaagaggatgatcaccggcccccagtggtgggccaggtgcaagcagatgaacgtgctggacagcttcatcaactactacgacagcgagaagcacgccgagaacgccgtgatcttcctgcacggcaacgccgctagcagctacctgtggaggcacgtggtgccccacatcgagcccgtggccaggtgcatcatccccgatctgatcggcatgggcaagagcggcaagagcggcaacggcagctacaggctgctggaccactacaagtacctgaccgcctggttcgagctcctgaacctgcccaagaagatcatcttcgtgggccacgactggggcgcctgcctggccttccactacagctacgagcaccaggacaagatcaaggccatcgtgcacgccgagagcgtggtggacgtgatcgagagctgggacgagtggccagacatcgaggaggacatcgccctgatcaagagcgaggagggcgagaagatggtgctggagaacaacttcttcgtggagaccatgctgcccagcaagatcatgagaaagctggagcccgaggagttcgccgcctacctggagcccttcaaggagaagggcgaggtgagaagacccaccctgagctggcccagagagatccccctggtgaagggcggcaagcccgacgtggtgcagatcgtgagaaactacaacgcctacctgagagccagcgacgacctgcccaagatgttcatcgagagcgaccccggcttcttcagcaacgccatcgtggagggcgccaagaagttccccaacaccgagttcgtgaaggtgaagggcctgcacttcagccaggaggacgcccccgacgagatgggcaagtacatcaagagcttcgtggagagagtgctgaagaacgagcagtaa

SEQ ID NO: 24 - DNA, 2706 bp, synthetic construct
  source 1..2706: mol_type = other DNA
atgtccgatatatactggatacaaattactgaagtttgctccttcgtcggatttatgctctcagttctagggaacagtacacttttagtactgctcagtggaaaatccatagatggaattggcacctatcggtacttgatgatcactttctgcgttttcagtttattatttacgatattagaggattttatcagaccgctgatgcatcactataacaataccataattgttttacaacgcaagcggtttcagttttctgattcaacggctagaatcttgacagtctcttactgcggctgtttcgcgatgtgcttcgtgatgttcgccgttcatttcatctatcgatatctagttgcttgtcacccgacaaaattgcactattttcgacccaaaaatttcattttctggctgtccggcatgttattcatagcaggaagctgggttgcaattgcatatgtcttttttcaagaagacctagaaaccaggacggatttggtatttattttgtcaacttgttataatttaacgccagatgatgtcggacatgtaccgtatgctttttacaaaactcaaggaaatacacgagtaattcgatgggataacatgattggagtaattcatcatatgatagttatgacaatctctataagtgccgttttctactttggcattaaaacctacactcgaataatgagtttcaagggaaaatcccagaaaacctccggaatggtgagcaagggcgaggagctgttcaccggggtggtgcccatcctggtcgagctggacggcgacgtaaacggccacaagttcagcgtgtccggcgagggcgagggcgatgccacctacggcaagctgaccctgaagttcatctgcaccaccggcaagctgcccgtgccctggcccaccctcgtgaccaccctgagctacggcgtgcagtgcttcagccgctaccccgaccacatgaagcagcacgacttcttcaagtccgccatgcccgaaggctacgtccaggagcgcaccatcttcttcaaggacgacggcaactacaagacccgcgccgaggtgaagttcgagggcgacaccctggtgaaccgcatcgagctgaagggcatcgacttcaaggaggacggcaacatcctggggcacaagctggagtacaactacaacagccacaacgtctatatcatggccgacaagcagaagaacggcatcaaggtgaacttcaagatccgccacaacatcgaggacggcagcgtgcagctcgccgaccactaccagcagaacacccccatcggcgacggccccgtgctgctgcccgacaaccactacctgagcacccagtccgccctgagcaaagaccccaacgagaagcgcgatcacatggtcctgctggagttcgtgaccgccgccgggatcactctcggcatggacgagctgtacaaggtcgacaaagaaatgcacacccaattgttcaaggccttggttctacagactatcatccctactacactaatgtacatcccgacaaccatgctctttgtcaccccattcgttggactcaacatcggctgttacggcaacatcactactgccaccgtccatttgtatcctggaattgacccagtcgttttgatctttataatccgagacttccggcaaacgattttaagaccattcagatgcttctaccgttcaaatagtgtcgaaaacactgccaccataaggcaataccagcagagcagctccaaaggatctagagaattcggtaccatggcttccaaggtgtacgaccccgagcaacgcaaacgcatgatcactgggcctcagtggtgggctcgctgcaagcaaatgaacgtgctggactccttcatcaactactatgattccgagaagcacgccgagaacgccgtgatttttctgcatggtaacgctgcctccagctacctgtggaggcacgtcgtgcctcacatcgagcccgtggctagatgcatcatccctgatctgatcggaatgggtaagtccggcaagagcgggaatggctcatatcgcctcctggatcactacaagtacctcaccgcttggttcgagctgctgaaccttccaaagaaaatcatctttgtgggccacgactggggggctgctctggcctttcactactcctacgagcaccaagacaagatcaaggccatcgtccatgctgagagtgtcgtggacgtgatcgagtcctgggacgagtggcctgacatcgaggaggatatcgccctgatcaagagcgaagagggcgagaaaatggtgcttgagaataacttcttcgtcgagaccgtgctcccaagcaagatcatgcggaaactggagcctgaggagttcgctgcctacctggagccattcaaggagaagggcgaggttagacggcctaccctctcctggcctcgcgagatccctctcgttaagggaggcaagcccgacgtcgtccagattgtccgcaactacaacgcctaccttcgggccagcgacgatctgcctaagatgttcatcgagtccgaccctgggttcttttccaacgctattgtcgagggagctaagaagttccctaacaccgagttcgtgaaggtgaagggcctccacttcagccaggaggacgctccagatgaaatgggtaagtacatcaagagcttcgtggagcgcgtgctgaagaacgagcagtaa

SEQ ID NO: 25 - protein, 889 aa, synthetic construct; identical to SEQ ID NO: 2

SEQ ID NO: 26 - protein, 889 aa, synthetic construct
MSGELWITLVDTADIVGVTLTFCVNIVLLGLLKTRGKNLGTYKYLMAFFSVFSIFYAIIEFILRPIMHIENTTFFLISRKRFNYSTKLGKINSAFYCACFATSFVVSGVYFVYRYFATCKPNLLRLFNLPTLLLWPLGCSVPVTMWASVSYFLYPDTEYTEAAVTNVLNNHYNWIKKENVSYIAYVYYQYENGVRHIYLKNLLGCFVHYFVMSMTFVVMFYCGYATWKTMNEHKDVSDRTMVSKGEELFTGVVPILVELDGDVNGHKFSVSGEGEGDATYGKLTLKFICTTGKLPVPWPTLVTTLSYGVQCFSRYPDHMKQHDFFKSAMPEGYVQERTIFFKDDGNYKTRAEVKFEGDTLVNRIELKGIDFKEDGNILGHKLEYNYNSHNVYIMADKQKNGIKVNFKIRHNIEDGSVQLADHYQQNTPIGDGPVLLPDNHYLSTQSALSKDPNEKRDHMVLLEFVTAAGITLGMDELYKRALQKQLFKALVLQTLIPTIFMYAPTGVMFIAPFFDVNLNANANFIVFCSFLYPGLDPLILILIIRDFRRTIFNFLCGKKNSVDESRSTTRANLSQVPTMTSKVYDPEQRKRMITGPQWWARCKQMNVLDSFINYYDSEKHAENAVIFLHGNAASSYLWRHVVPHIEPVARCIIPDLIGMGKSGKSGNGSYRLLDHYKYLTAWFELLNLPKKIIFVGHDWGAALAFHYSYEHQDKIKAIVHAESVVDVIESWDEWPDIEEDIALIKSEEGEKMVLENNFFVETVLPSKIMRKLEPEEFAAYLEPFKEKGEVRRPTLSWPREIPLVKGGKPDVVQIVRNYNAYLRASDDLPKMFIESDPGFFSNAIVEGAKKFPNTEFVKVKGLHFSQEDAPDEMGKYIKSFVERVLKNEQ

SEQ ID NO: 27 - protein, 897 aa, synthetic construct
MGSGQLWLALVDAADMVGFTLTISINIILLGLIRTRGKTLGTYKYLMSFFSFFSIFYAIVESILRPIMHIENTTFFLISRKRFDYSTRLGKINSAFYCACFATSFVLSAVHFVYRYFAACKPNLLRLFNLPHLLLWPLMCSIPVTAWASVSYFLYPDTEYTEAAVTYVLKTHYEVIKKENVSYIAYVYYQYENGERHIYIKNLLGCFVHYFVMSMTFVVVFYCGFSTWWTIREHRGASDRTMVSKGEELFTGVVPILVELDGDVNGHKFSVSGEGEGDATYGKLTLKFICTTGKLPVPWPTLVTTLTYGVQCFSRYPDHMKQHDFFKSAMPEGYVQERTIFFKDDGNYKTRAEVKFEGDTLVNRIELKGIDFKEDGNILGHKLEYNYNSHNVYIMADKQKNGIKVNFKIRHNIEDGSVQLADHYQQNTPIGDGPVLLPDNHYLSTQSALSKDPNEKRDHMVLLEFVTAAGITLGMDELYKRHLHRQLFKALVFQTLVPSIFMYIPTGVMFIAPFFDINLNANANFIVFCSFLYPGLDPLILIFIIREFRVTILNIIRGNERGNAVGEAYSTSRIKSSQPAAVNLSGMTSKVYDPEQRKRMITGPQWWARCKQMNVLDSFINYYDSEKHAENAVIFLHGNAASSYLWRHVVPHIEPVARCIIPDLIGMGKSGKSGNGSYRLLDHYKYLTAWFELLNLPKKIIFVGHDWGAALAFHYSYEHQDKIKAIVHAESVVDVIESWDEWPDIEEDIALIKSEEGEKMVLENNFFVETVLPSKIMRKLEPEEFAAYLEPFKEKGEVRRPTLSWPREIPLVKGGKPDVVQIVRNYNAYLRASDDLPKMFIESDPGFFSNAIVEGAKKFPNTEFVKVKGLHFSQEDAPDEMGKYIKSFVERVLKNEQ

SEQ ID NO: 28 - protein, 901 aa, synthetic construct
MSDRHWLDITTYSDHIGFTISTIANFVLILLLVFRPTKSYGSYKYLMITFCVFSLFYTSIETFLRPLIHIYDNTIFVIQRKRFQYSEGTARAISSTYCGCYAMSFTLFAVHFVYRYYAACKPDNLRYFQGCYFVAWVFGAMAVAASWGFAAFILYPETERTRTALIHVIQTSYELDPEWVGNVPYSYWRTENGVEYLNPRNVIGIFQHGVIMILSFGTVFYCGFNTYKTLNGSLGVSEKTSGMVSKGEELFTGVVPILVELDGDVNGHKFSVSGEGEGDATYGKLTLKFICTTGKLPVPWPTLVTTLSYGVQCFSRYPDHMKQHDFFKSAMPEGYVQERTIFFKDDGNYKTRAEVKFEGDTLVNRIELKGIDFKEDGNILGHKLEYNYNSHNVYIMADKQKNGIKVNFKIRHNIEDGSVQLADHYQQNTPIGDGPVLLPDNHYLSTQSALSKDPNEKRDHMVLLEFVTAAGITLGMDELYKVDKEMHTQLFKALVLQTIIPTTLMYIPTTMLFVTPFVGLNIGCYGNITTATVHLYPGIDPVVLIFIIRDFRQTILRPFRCFYRSNSVENTATIRQYQQSSSKGSREFGTMTSKVYDPEQRKRMITGPQWWARCKQMNVLDSFINYYDSEKHAENAVIFLHGNAASSYLWRHVVPHIEPVARCIIPDLIGMGKSGKSGNGSYRLLDHYKYLTAWFELLNLPKKIIFVGHDWGAALAFHYSYEHQDKIKAIVHAESVVDVIESWDEWPDIEEDIALIKSEEGEKMVLENNFFVETVLPSKIMRKLEPEEFAAYLEPFKEKGEVRRPTLSWPREIPLVKGGKPDVVQIVRNYNAYLRASDDLPKMFIESDPGFFSNAIVEGAKKFPNTEFVKVKGLHFSQEDAPDEMGKYIKSFVERVLKNEQ

SEQ ID NO: 29 - protein, 908 aa, synthetic construct
MSDIYWIQITEVCSFVGFMLSVLGNSTLLVLLSGKSIDGIGTYRYLMITFCVFSLLFTILEDFIRPLMHHYNNTIIVLQRKRFQFSDSTARILTVSYCGCFAMCFVMFAVHFIYRYLVACHPTKLHYFRPKNFIFWLSGMLFIAGSWVAIAYVFFQEDLETRTDLVFILSTCYNLTPDDVGHVPYAFYKTQGNTRVIRWDNMIGVIHHMIVMTISISAVFYFGIKTYTRIMSFKGKSQKTSGMVSKGEELFTGVVPILVELDGDVNGHKFSVSGEGEGDATYGKLTLKFICTTGKLPVPWPTLVTTLSYGVQCFSRYPDHMKQHDFFKSAMPEGYVQERTIFFKDDGNYKTRAEVKFEGDTLVNRIELKGIDFKEDGNILGHKLEYNYNSHNVYIMADKQKNGIKVNFKIRHNIEDGSVQLADHYQQNTPIGDGPVLLPDNHYLSTQSALSKDPNEKRDHMVLLEFVTAAGITLGMDELYKVDKDLQNQFFTALVAQTVVPLIFMFIPNMVLTTAALIDGTFGSWANITVVMNHLYPAADPFVILFIIKGFRNSIRNVIYRCTKTKKASVSSVVRGIEAQSKKQSFSRVDISREFGTMTSKVYDPEQRKRMITGPQWWARCKQMNVLDSFINYYDSEKHAENAVIFLHGNAASSYLWRHVVPHIEPVARCIIPDLIGMGKSGKSGNGSYRLLDHYKYLTAWFELLNLPKKIIFVGHDWGAALAFHYSYEHQDKIKAIVHAESVVDVIESWDEWPDIEEDIALIKSEEGEKMVLENNFFVETVLPSKIMRKLEPEEFAAYLEPFKEKGEVRRPTLSWPREIPLVKGGKPDVVQIVRNYNAYLRASDDLPKMFIESDPGFFSNAIVEGAKKFPNTEFVKVKGLHFSQEDAPDEMGKYIKSFVERVLKNEQ

SEQ ID NO: 30 - protein, 901 aa, synthetic construct
MSDIYWIQITEVCSFVGFMLSVLGNSTLLVLLSGKSIDGIGTYRYLMITFCVFSLLFTILEDFIRPLMHHYNNTIIVLQRKRFQFSDSTARILTVSYCGCFAMCFVMFAVHFIYRYLVACHPTKLHYFRPKNFIFWLSGMLFIAGSWVAIAYVFFQEDLETRTDLVFILSTCYNLTPDDVGHVPYAFYKTQGNTRVIRWDNMIGVIHHMIVMTISISAVFYFGIKTYTRIMSFKGKSQKTSGMVSKGEELFTGVVPILVELDGDVNGHKFSVSGEGEGDATYGKLTLKFICTTGKLPVPWPTLVTTLSYGVQCFSRYPDHMKQHDFFKSAMPEGYVQERTIFFKDDGNYKTRAEVKFEGDTLVNRIELKGIDFKEDGNILGHKLEYNYNSHNVYIMADKQKNGIKVNFKIRHNIEDGSVQLADHYQQNTPIGDGPVLLPDNHYLSTQSALSKDPNEKRDHMVLLEFVTAAGITLGMDELYKVDKEMHTQLFKALVLQTIIPTTLMYIPTTMLFVTPFVGLNIGCYGNITTATVHLYPGIDPVVLIFIIRDFRQTILRPFRCFYRSNSVENTATIRQYQQSSSKGSREFGTMTSKVYDPEQRKRMITGPQWWARCKQMNVLDSFINYYDSEKHAENAVIFLHGNAASSYLWRHVVPHIEPVARCIIPDLIGMGKSGKSGNGSYRLLDHYKYLTAWFELLNLPKKIIFVGHDWGAALAFHYSYEHQDKIKAIVHAESVVDVIESWDEWPDIEEDIALIKSEEGEKMVLENNFFVETVLPSKIMRKLEPEEFAAYLEPFKEKGEVRRPTLSWPREIPLVKGGKPDVVQIVRNYNAYLRASDDLPKMFIESDPGFFSNAIVEGAKKFPNTEFVKVKGLHFSQEDAPDEMGKYIKSFVERVLKNEQ

SEQ ID NO: 31 - protein, 890 aa, synthetic construct
MTDQHWVIITDIAGPIGFSMSIFSNSILLFLIFSHSSPIKGPYKRMLIVFCIFTVFYSFVEVMLQPLIHIYDDTLFLIHRKRIDLPKWLTRLVPTTYCWCYAMSFSLFALQFLYRYVAVCKPQYVDLFVGCHFYAWVVLILSLATSWGLTAAFMFPQTDRTTEIFLHIIYSSYDLEPYWTDYVAYKYFDTDENNVRWVNVLSFFGVLQHGIVITLSFGTLYYCGINTYLKIKKHTGTSNRTSGMVSKGEELFTGVVPILVELDGDVNGHKFSVSGEGEGDATYGKLTLKFICTTGKLPVPWPTLVTTLSYGVQCFSRYPDHMKQHDFFKSAMPEGYVQERTIFFKDDGNYKTRAEVKFEGDTLVNRIELKGIDFKEDGNILGHKLEYNYNSHNVYIMADKQKNGIKVNFKIRHNIEDGSVQLADHYQQNTPIGDGPVLLPDNHYLSTQSALSKDPNEKRDHMVLLEFVTAAGITLGMDELYKVDRCIQLQLFRALVAQTILPMFMMYIPVGFMFACPYFDLQLGAYTNYQTVMAQLYPGIDPFVMLFLIDSYRITIFGWLCPRFVYVKPMHSTYTLTSRMTSKVYDPEQRKRMITGPQWWARCKQMNVLDSFINYYDSEKHAENAVIFLHGNAASSYLWRHVVPHIEPVARCIIPDLIGMGKSGKSGNGSYRLLDHYKYLTAWFELLNLPKKIIFVGHDWGAALAFHYSYEHQDKIKAIVHAESVVDVIESWDEWPDIEEDIALIKSEEGEKMVLENNFFVETVLPSKIMRKLEPEEFAAYLEPFKEKGEVRRPTLSWPREIPLVKGGKPDVVQIVRNYNAYLRASDDLPKMFIESDPGFFSNAIVEGAKKFPNTEFVKVKGLHFSQEDAPDEMGKYIKSFVERVLKNEQ

SEQ ID NO: 32 - protein, 906 aa, synthetic construct
MTDRRWVAITDIAGPIGFTMSIFSNSVLLSLIFSSSSPIKGAYKNMLIVLCIFTMFYSFVEIMLQPLIHIYDDTLFLIHRKRFDLSKGITRLIPTTYCWCYAMSFSLFALQFLYRYVAVCKPHLVVFFTGCYFYYWLALILSLATSWGLTAAFMFPQTNRTTESFNYVIKTSYDLDPYWTDYVAYKYFDTDENHVRWVNVLSLFGVLQHGLVITLSFGTLFYCGIKTYLSITEHVGMSSKTSGMVSKGEELFTGVVPILVELDGDVNGHKFSVSGEGEGDATYGKLTLKFICTTGKLPVPWPTLVTTLSYGVQCFSRYPDHMKQHDFFKSAMPEGYVQERTIFFKDDGNYKTRAEVKFEGDTLVNRIELKGIDFKEDGNILGHKLEYNYNSHNVYIMADKQKNGIKVNFKIRHNIEDGSVQLADHYQQNTPIGDGPVLLPDNHYLSTQSALSKDPNEKRDHMVLLEFVTAAGITLGMDELYKVDRSLQLQLFRALVAQTCLPMLMMYMPIGFMFSCPYFDLQLGAVTNYQTVMAQLYPGIDPFMLLFLINAYRKTVLSLICPNFIQKKYVQTATTRDGTDASATMNSVKSTQLGTMTSKVYDPEQRKRMITGPQWWARCKQMNVLDSFINYYDSEKHAENAVIFLHGNAASSYLWRHVVPHIEPVARCIIPDLIGMGKSGKSGNGSYRLLDHYKYLTAWFELLNLPKKIIFVGHDWGAALAFHYSYEHQDKIKAIVHAESVVDVIESWDEWPDIEEDIALIKSEEGEKMVLENNFFVETVLPSKIMRKLEPEEFAAYLEPFKEKGEVRRPTLSWPREIPLVKGGKPDVVQIVRNYNAYLRASDDLPKMFIESDPGFFSNAIVEGAKKFPNTEFVKVKGLHFSQEDAPDEMGKYIKSFVERVLKNEQ

SEQ ID NO: 33 - DNA, 2670 bp, synthetic construct; identical to SEQ ID NO: 1
  source 1..2670: mol_type = other DNA

SEQ ID NO: 34 - DNA, 2670 bp, synthetic construct
  source 1..2670: mol_type = other DNA
atgtcgggagaattgtggattaccctagttgacacagcggacattgtcggcgtcaccctcaccttctgtgtcaacattgttcttctcggacttctgaaaacacgtggaaaaaacttgggcacttataaatatctcatggcgtttttctcagtattctcgattttttacgccatcatcgagttcatattacgacctataatgcatattgagaacaccactttctttttgatctcaaggaaaagattcaactactccaccaaacttggaaaaatcaactctgcgttttactgtgcttgttttgccaccagttttgttgtctcaggagtttattttgtttatcgatattttgcaacttgcaaaccgaatctacttcgtttgttcaacttgccaactcttctactttggccacttggttgcagtgtacccgtgacaatgtgggctagtgtctcatattttttgtatccagataccgagtacacggaagcggctgtcaccaatgtactaaataaccactataactggatcaaaaaggagaatgtatcgtacattgcatacgtctattaccaatacgaaaacggagtaaggcatatctacctcaaaaacttgcttggatgctttgttcattactttgtcatgtcgatgacgtttgttgtgatgttctactgcggatatgccacgtggaaaactatgaatgaacacaaggatgtatctgatagaactatggtgagcaagggcgaggagctgttcaccggggtggtgcccatcctggtcgagctggacggcgacgtaaacggccacaagttcagcgtgtccggcgagggcgagggcgatgccacctacggcaagctgaccctgaagttcatctgcaccaccggcaagctgcccgtgccctggcccaccctcgtgaccaccctgagctacggcgtgcagtgcttcagccgctaccccgaccacatgaagcagcacgacttcttcaagtccgccatgcccgaaggctacgtccaggagcgcaccatcttcttcaaggacgacggcaactacaagacccgcgccgaggtgaagttcgagggcgacaccctggtgaaccgcatcgagctgaagggcatcgacttcaaggaggacggcaacatcctggggcacaagctggagtacaactacaacagccacaacgtctatatcatggccgacaagcagaagaacggcatcaaggtgaacttcaagatccgccacaacatcgaggacggcagcgtgcagctcgccgaccactaccagcagaacacccccatcggcgacggccccgtgctgctgcccgacaaccactacctgagcacccagtccgccctgagcaaagaccccaacgagaagcgcgatcacatggtcctgctggagttcgtgaccgccgccgggatcactctcggcatggacgagctgtacaagcgagcgctacagaaacaacttttcaaagctttagttcttcagacactcatcccaactatcttcatgtacgccccaactggagtcatgttcatcgcaccgttttttgacgtgaatttgaatgcaaacgccaatttcattgtgttttgctcatttctgtacccgggactcgatccactcattctgattttgatcattcgtgatttccgaagaacaatattcaatttcttgtgtggaaagaaaaacagtgttgatgaatcccgctcgacaacaagagccaatttgtctcaagttccgacgatgaccagcaaggtgtacgaccccgagcagaggaagaggatgatcaccggcccccagtggtgggccaggtgcaagcagatgaacgtgctggacagcttcatcaactactacgacagcgagaagcacgccgagaacgccgtgatcttcctgcacggcaacgccgctagcagctacctgtggaggcacgtggtgccccacatcgagcccgtggccaggtgcatcatccccgatctgatcggcatgggcaagagcggcaagagcggcaacggcagctacaggctgctggaccactacaagtacctgaccgcctggttcgagctcctgaacctgcccaagaagatcatcttcgtgggccacgactggggcgccgccctggccttccactacagctacgagcaccaggacaagatcaaggccatcgtgcacgccgagagcgtggtggacgtgatcgagagctgggacgagtggccagacatcgaggaggacatcgccctgatcaagagcgaggagggcgagaagatggtgctggagaacaacttcttcgtggagaccgtgctgcccagcaagatcatgagaaagctggagcccgaggagttcgccgcctacctggagcccttcaaggagaagggcgaggtgagaagacccaccctgagctggcccagagagatccccctggtgaagggcggcaagcccgacgtggtgcagatcgtgagaaactacaacgcctacctgagagccagcgacgacctgcccaagatgttcatcgagagcgaccccggcttcttcagcaacgccatcgtggagggcgccaagaagttccccaacaccgagttcgtgaaggtgaagggcctgcacttcagccaggaggacgcccccgacgagatgggcaagtacatcaagagcttcgtggagagagtgctgaagaacgagcagtaa

SEQ ID NO: 35 - DNA, 2714 bp, synthetic construct
  source 1..2714: mol_type = other DNA
atgtctgaccgtcattggctcgacatcaccacctactcagaccacattgggtttacgatttccaccatcgccaatttcgttctgatccttctgctagtcttccgaccgaccaaatcatacggttcatacaagtacctgatgatcacattctgcgtgttcagcctcttttacacctccattgaaacttttttgagacctctcatccatatctacgacaatacgatcttcgtgattcagcgcaagagattccagtactccgagggtaccgctagagccatttcatcgacctactgcggctgctacgccatgagcttcaccctgttcgccgtccactttgtctaccgttactatgcggcttgcaaacccgacaacctccgttacttccaaggatgctactttgtcgcatgggtattcggagcaatggcggtggcggcgagctgggggttcgcagcgtttattctgtacccggagaccgagaggaccaggacggcgttgatacacgtcatacaaacatcctatgagctggatcccgagtgggtgggaaatgttccatatagctattggcgcacagaaaacggagtggaatacctgaatcctcgcaacgtcatcgggatctttcaacacggcgtcatcatgatcctctccttcggaacagtcttctactgcggattcaacacttataagactttgaacggaagtctgggggtgtctgaaaaaacatccggaatggtgagcaagggcgaggagctgttcaccggggtggtgcccatcctggtcgagctggacggcgacgtaaacggccacaagttcagcgtgtccggcgagggcgagggcgatgccacctacggcaagctgaccctgaagttcatctgcaccaccggcaagctgcccgtgccctggcccaccctcgtgaccaccctgagctacggcgtgcagtgcttcagccgctaccccgaccacatgaagcagcacgacttcttcaagtccgccatgcccgaaggctacgtccaggagcgcaccatcttcttcaaggacgacggcaactacaagacccgcgccgaggtgaagttcgagggcgacaccctggtgaaccgcatcgagctgaagggcatcgacttcaaggaggacggcaacatcctggggcacaagctggagtacaactacaacagccacaacgtctatatcatggccgacaagcagaagaacggcatcaaggtgaacttcaagatccgccacaacatcgaggacggcagcgtgcagctcgccgaccactaccagcagaacacccccatcggcgacggccccgtgctgctgcccgacaaccactacctgagcacccagtccgccctgagcaaagaccccaacgagaagcgcgatcacatggtcctgctggagttcgtgaccgccgccgggatcactctcggcatggacgagctgtacaaggtcgacaaagaaatgcacacccaattgttcaaggccttggttctacagactatcatccctactacactaatgtacatcccgacaaccatgctctttgtcaccccattcgttggactcaacatcggctgttacggcaacatcactactgccaccgtccatttgtatcctggaattgacccagtcgttttgatctttataatccgagacttccggcaaacgattttaagaccattcagatgcttctaccgttcaaatagtgtcgaaaacactgccaccataaggcaataccagcagagcagctccaaaggatctagagaattcggtaccatgaccagcaaggtgtacgaccccgagcagaggaagaggatgatcaccggcccccagtggtgggccaggtgcaagcagatgaacgtgctggacagcttcatcaactactacgacagcgagaagcacgccgagaacgccgtgatcttcctgcacggcaacgccgctagcagctacctgtggaggcacgtggtgccccacatcgagcccgtggccaggtgcatcatccccgatctgatcggcatgggcaagagcggcaagagcggcaacggcagctacaggctgctggaccactacaagtacctgaccgcctggttcgagctcctgaacctgcccaagaagatcatcttcgtgggccacgactggggcgccgccctggccttccactacagctacgagcaccaggacaagatcaaggccatcgtgcacgccgagagcgtggtggacgtgatcgagagctgggacgagtggccagacatcgaggaggacatcgccctgatcaagagcgaggagggcgagaagatggtgctggagaacaacttcttcgtggagaccgtgctgcccagcaagatcatgagaaagctggagcccgaggagttcgccgcctacctggagcccttcaaggagaagggcgaggtgagaagacccaccctgagctggcccagagagatccccctggtgaagggcggcaagcccgacgtggtgcagatcgtgagaaactacaacgcctacctgagagccagcgacgacctgcccaagatgttcatcgagagcgaccccggcttcttcagcaacgccatcgtggagggcgccaagaagttccccaacaccgagttcgtgaaggtgaagggcctgcacttcagccaggaggacgcccccgacgagatgggcaagtacatcaagagcttcgtggagagagtgctgaagaacgagcagtaagcggccgc

SEQ ID NO: 36 - DNA, 2714 bp, synthetic construct; identical to SEQ ID NO: 35
  source 1..2714: mol_type = other DNA

SEQ ID NO: 37 - DNA, 2714 bp, synthetic construct; identical to SEQ ID NO: 35
  source 1..2714: mol_type = other DNA

SEQ ID NO: 38 - DNA, 2714 bp, synthetic construct; identical to SEQ ID NO: 35
  source 1..2714: mol_type = other DNA

SEQ ID NO: 39 - DNA, 2673 bp, synthetic construct
  source 1..2673: mol_type = other DNA
atgactgatcaacactgggttattatcacagatattgctggtccaatcggattttcaatgtccattttttcaaactctattcttttgtttttgatattttcacattcatctccaataaaaggtccatacaaacgaatgctcatagtattttgcatatttaccgtattctactcatttgtcgaagtcatgcttcagccactaatccatatttacgacgacactttatttttgattcatcgaaagagaatagacttgccaaaatggttaacacgtttggttcctactacctattgttggtgttacgcaatgagtttttccttgtttgcattacaatttttatatagatatgtggcagtatgcaaaccgcaatatgttgatctttttgtcggatgtcacttttatgcttgggtagttttgatcttatcactagccacgagctggggactcactgcagctttcatgttcccacaaaccgaccgaacaactgaaatttttttgcacataatttatagttcatatgacttggagccttattggacagattatgttgcttataaatactttgatactgatgagaataatgtgagatgggtcaatgttcttagttttttcggtgtccttcagcacgggattgtaattactctaagttttggcaccctttattattgtggcatcaacacgtatctcaaaataaaaaaacacactggaacatcaaacagaacttccggaatggtgagcaagggcgaggagctgttcaccggggtggtgcccatcctggtcgagctggacggcgacgtaaacggccacaagttcagcgtgtccggcgagggcgagggcgatgccacctacggcaagctgaccctgaagttcatctgcaccaccggcaagctgcccgtgccctggcccaccctcgtgaccaccctgagctacggcgtgcagtgcttcagccgctaccccgaccacatgaagcagcacgacttcttcaagtccgccatgcccgaaggctacgtccaggagcgcaccatcttcttcaaggacgacggcaactacaagacccgcgccgaggtgaagttcgagggcgacaccctggtgaaccgcatcgagctgaagggcatcgacttcaaggaggacggcaacatcctggggcacaagctggagtacaactacaacagccacaacgtctatatcatggccgacaagcagaagaacggcatcaaggtgaacttcaagatccgccacaacatcgaggacggcagcgtgcagctcgccgaccactaccagcagaacacccccatcggcgacggccccgtgctgctgcccgacaaccactacctgagcacccagtccgccctgagcaaagaccccaacgagaagcgcgatcacatggtcctgctggagttcgtgaccgccgccgggatcactctcggcatggacgagctgtacaaggtcgaccgatgtattcaactacaacttttcagagctctggttgcacagacaattttaccaatgttcatgatgtatattcccgttggtttcatgtttgcatgtccatattttgacttgcaattaggtgcatacaccaattatcaaacagtcatggcacaactttatccgggaatcgacccatttgtgatgctgtttttgatagattcttatagaataacaatatttggatggttatgtccaagatttgtttatgtaaagccgatgcattccacatacaccctaacttctagaatgaccagcaaggtgtacgaccccgagcagaggaagaggatgatcaccggcccccagtggtgggccaggtgcaagcagatgaacgtgctggacagcttcatcaactactacgacagcgagaagcacgccgagaacgccgtgatcttcctgcacggcaacgccgctagcagctacctgtggaggcacgtggtgccccacatcgagcccgtggccaggtgcatcatccccgatctgatcggcatgggcaagagcggcaagagcggcaacggcagctacaggctgctggaccactacaagtacctgaccgcctggttcgagctcctgaacctgcccaagaagatcatcttcgtgggccacgactggggcgccgccctggccttccactacagctacgagcaccaggacaagatcaaggccatcgtgcacgccgagagcgtggtggacgtgatcgagagctgggacgagtggccagacatcgaggaggacatcgccctgatcaagagcgaggagggcgagaagatggtgctggagaacaacttcttcgtggagaccgtgctgcccagcaagatcatgagaaagctggagcccgaggagttcgccgcctacctggagcccttcaaggagaagggcgaggtgagaagacccaccctgagctggcccagagagatccccctggtgaagggcggcaagcccgacgtggtgcagatcgtgagaaactacaacgcctacctgagagccagcgacgacctgcccaagatgttcatcgagagcgaccccggcttcttcagcaacgccatcgtggagggcgccaagaagttccccaacaccgagttcgtgaaggtgaagggcctgcacttcagccaggaggacgcccccgacgagatgggcaagtacatcaagagcttcgtggagagagtgctgaagaacgagcagtaa

SEQ ID NO: 40 - DNA, 2729 bp, synthetic construct
  source 1..2729: mol_type = other DNA
atgaccgatcgtcgctgggtcgctattacggacattgccggaccgattgggttcacaatgtcaattttttcgaactcggtgctgttatcgttgatattctcaagcagctctccaattaaaggagcttacaaaaatatgttgatagtgttgtgtatattcactatgttctactcttttgttgaaataatgcttcaaccgttgattcatatttatgatgacacgctgttcttgatccaccggaaaagatttgacctgtctaaaggaattacacgtttgatacctacaacatattgttggtgttatgcaatgagtttctcattattcgccctccagtttttgtacagatatgtggcagtttgcaaacctcacttagttgttttttttactggatgctatttctattattggttggcactcatcttatcacttgctacaagttgggggcttactgcagcttttatgttcccgcaaaccaatcgaacaactgaaagcttcaactacgtaataaaaacttcttatgacttagatccttattggacggattatgttgcctataaatattttgacaccgatgagaatcatgtgagatgggtgaatgttcttagtttatttggagtcttgcagcacggattagtaattacgttgagttttggaaccttattctactgtggaattaaaacttatctcagcattactgaacatgttggaatgtccagcaagacctccggaatggtgagcaagggcgaggagctgttcaccggggtggtgcccatcctggtcgagctggacggcgacgtaaacggccacaagttcagcgtgtccggcgagggcgagggcgatgccacctacggcaagctgaccctgaagttcatctgcaccaccggcaagctgcccgtgccctggcccaccctcgtgaccaccctgagctacggcgtgcagtgcttcagccgctaccccgaccacatgaagcagcacgacttcttcaagtccgccatgcccgaaggctacgtccaggagcgcaccatcttcttcaaggacgacggcaactacaagacccgcgccgaggtgaagttcgagggcgacaccctggtgaaccgcatcgagctgaagggcatcgacttcaaggaggacggcaacatcctggggcacaagctggagtacaactacaacagccacaacgtctatatcatggccgacaagcagaagaacggcatcaaggtgaacttcaagatccgccacaacatcgaggacggcagcgtgcagctcgccgaccactaccagcagaacacccccatcggcgacggccccgtgctgctgcccgacaaccactacctgagcacccagtccgccctgagcaaagaccccaacgagaagcgcgatcacatggtcctgctggagttcgtgaccgccgccgggatcactctcggcatggacgagctgtacaaggtcgaccgaagtcttcaacttcaactattccgtgctttagttgctcagacatgtcttccaatgctcatgatgtacatgccaataggattcatgttttcttgcccttactttgatttgcaacttggagcagtcacaaactatcaaaccgtcatggcacagttatacccaggaatcgacccatttatgttgctatttcttattaacgcctacagaaagacagtgttaagcttgatctgtcctaattttatccagaaaaaatatgttcaaacggcaactactcgtgatggcacagatgcctcggcaacaatgaattctgttaaatctacacagttaggtaccatgaccagcaaggtgtacgaccccgagcagaggaagaggatgatcaccggcccccagtggtgggccaggtgcaagcagatgaacgtgctggacagcttcatcaactactacgacagcgagaagcacgccgagaacgccgtgatcttcctgcacggcaacgccgctagcagctacctgtggaggcacgtggtgccccacatcgagcccgtggccaggtgcatcatccccgatctgatcggcatgggcaagagcggcaagagcggcaacggcagctacaggctgctggaccactacaagtacctgaccgcctggttcgagctcctgaacctgcccaagaagatcatcttcgtgggccacgactggggcgccgccctggccttccactacagctacgagcaccaggacaagatcaaggccatcgtgcacgccgagagcgtggtggacgtgatcgagagctgggacgagtggccagacatcgaggaggacatcgccctgatcaagagcgaggagggcgagaagatggtgctggagaacaacttcttcgtggagaccgtgctgcccagcaagatcatgagaaagctggagcccgaggagttcgccgcctacctggagcccttcaaggagaagggcgaggtgagaagacccaccctgagctggcccagagagatccccctggtgaagggcggcaagcccgacgtggtgcagatcgtgagaaactacaacgcctacctgagagccagcgacgacctgcccaagatgttcatcgagagcgaccccggcttcttcagcaacgccatcgtggagggcgccaagaagttccccaacaccgagttcgtgaaggtgaagggcctgcacttcagccaggaggacgcccccgacgagatgggcaagtacatcaagagcttcgtggagagagtgctgaagaacgagcagtaagcggccgc

SEQ ID NO: 41 - protein, 346 aa, Caenorhabditis elegans
MSGQLWLALVDAADMVGFTLTISINIILLGLIRTRGKTLGTYKYLMSFFSFFSIFYAIVESILRPIMHIENTTFFLISRKRFDYSTRLGKINSAFYCACFATSFVLSAVHFVYRYFAACKPNLLRLFNLPHLLLWPLMCSIPVTAWASVSYFLYPDTEYTEAAVTYVLKTHYEVIKKENVSYIAYVYYQYENGERHIYIKNLLGCFVHYFVMSMTFVVVFYCGFSTWWTIREHRGASDRTRHLHRQLFKALVFQTLVPSIFMYIPTGVMFIAPFFDINLNANANFIVFCSFLYPGLDPLILIFIIREFRVTILNIIRGNERGNAVGEAYSTSRIKSSQPAAVNLSG

SEQ ID NO: 42 - protein, 341 aa, Caenorhabditis elegans
MSDRHWLDITTYSDHIGFTISTIANFVLILLLVFRPTKSYGSYKYLMITFCVFSLFYTSIETFLRPLIHIYDNTIFVIQRKRFQYSEGTARAISSTYCGCYAMSFTLFAVHFVYRYYAACKPDNLRYFQGCYFVAWVFGAMAVAASWGFAAFILYPETERTRTALIHVIQTSYELDPEWVGNVPYSYWRTENGVEYLNPRNVIGIFQHGVIMILSFGTVFYCGFNTYKTLNGSLGVSEKTKEMHTQLFKALVLQTIIPTTLMYIPTTMLFVTPFVGLNIGCYGNITTATVHLYPGIDPVVLIFIIRDFRQTILRPFRCFYRSNSVENTATIRQYQQSSSKG

SEQ ID NO: 43 - protein, 351 aa, synthetic construct
MSDRHWLDITTYSDHIGFTISTIANFVLILLLVFRPTKSYGSYKYLMITFCVFSLFYTSIETFLRPLIHIYDNTIFVIQRKRFQYSEGTARAISSTYCGCYAMSFTLFAVHFVYRYYAACKPDNLRYFQGCYFVAWVFGAMAVAASWGFAAFILYPETERTRTALIHVIQTSYELDPEWVGNVPYSYWRTENGVEYLNPRNVIGIFQHGVIMILSFGTVFYCGFNTYKTLNGSLGVSEKTSGVDKEMHTQLFKALVLQTIIPTTLMYIPTTMLFVTPFVGLNIGCYGNITTATVHLYPGIDPVVLIFIIRDFRQTILRPFRCFYRSNSVENTATIRQYQQSSSKGSREFGT

SEQ ID NO: 44 - DNA, 1041 bp, Caenorhabditis elegans
  source 1..1041: mol_type = genomic DNA
atgtctggtcaattatggttggccctcgtggatgctgccgatatggtaggattcactctcacgatctccatcaacatcattctactggggctgattagaacacgtggaaaaacgttgggaacgtacaaatacttgatgagcttcttctcgttcttctcaatcttttatgcaatcgttgaatctattttgagaccaataatgcatatcgaaaacacgacgttctttctgatttctcggaaacgcttcgattactcaactcgccttggtaaaatcaactctgctttctactgtgcttgttttgccacgagttttgtcctgtctgcggtacactttgtgtatcggtactttgccgcttgcaaaccgaatctgctacgcttgtttaaccttccgcatcttttactgtggcctttgatgtgttcgattcctgtgactgcgtgggcaagtgtttcttactttttgtacccagacaccgagtacactgaagcagcagttacatatgttctgaaaacacactacgaggtgatcaaaaaagaaaatgtatcttatatcgcatacgtatactatcaatatgaaaatggggagcgtcacatctacataaaaaatttgcttggctgctttgtacactacttcgttatgtcaatgacatttgtagttgtgttttactgcggattttctacatggtggacgattcgtgagcatcgtggagcatctgataggacacgtcacctgcatagacaattgtttaaggcacttgtatttcaaacccttgttccatcaatatttatgtacatcccaactggtgtcatgttcatcgctccctttttcgacatcaacctgaatgccaatgcaaacttcatcgttttttgctcatttctctatccaggtcttgacccactaattctcatttttatcattcgcgaattcagggtcactattttgaatatcatcagaggaaatgagcggggaaatgctgttggcgaagcatactcaacttctcgaataaaatcatcacaacctgcagctgttaatctttctggataa

SEQ ID NO: 45 - DNA, 1026 bp, Caenorhabditis elegans
  source 1..1026: mol_type = genomic DNA
atgtctgaccgtcattggctcgacatcaccacctactcagaccacattgggtttacgatttccaccatcgccaatttcgttctgatccttctgctagtcttccgaccgaccaaatcatacggttcatacaagtacctgatgatcacattctgcgtgttcagcctcttttacacctccattgaaacttttttgagacctctcatccatatctacgacaatacgatcttcgtgattcagcgcaagagattccagtactccgagggtaccgctagagccatttcatcgacctactgcggctgctacgccatgagcttcaccctgttcgccgtccactttgtctaccgttactatgcggcttgcaaacccgacaacctccgttacttccaaggatgctactttgtcgcatgggtattcggagcaatggcggtggcggcgagctgggggttcgcagcgtttattctgtacccggagaccgagaggaccaggacggcgttgatacacgtcatacaaacatcctatgagctggatcccgagtgggtgggaaatgttccatatagctattggcgcacagaaaacggagtggaatacctgaatcctcgcaacgtcatcgggatctttcaacacggcgtcatcatgatcctctccttcggaacagtcttctactgcggattcaacacttataagactttgaacggaagtctgggggtgtctgaaaaaacaaaagaaatgcacacccaattgttcaaggccttggttctacagactatcatccctactacactaatgtacatcccgacaaccatgctctttgtcaccccattcgttggactcaacatcggctgttacggcaacatcactactgccaccgtccatttgtatcctggaattgacccagtcgttttgatctttataatccgagacttccggcaaacgattttaagaccattcagatgcttctaccgttcaaatagtgtcgaaaacactgccaccataaggcaataccagcagagcagctccaaaggataa

SEQ ID NO: 46 - DNA, 1056 bp, synthetic construct
  source 1..1056: mol_type = other DNA
atgtctgaccgtcattggctcgacatcaccacctactcagaccacattgggtttacgatttccaccatcgccaatttcgttctgatccttctgctagtcttccgaccgaccaaatcatacggttcatacaagtacctgatgatcacattctgcgtgttcagcctcttttacacctccattgaaacttttttgagacctctcatccatatctacgacaatacgatcttcgtgattcagcgcaagagattccagtactccgagggtaccgctagagccatttcatcgacctactgcggctgctacgccatgagcttcaccctgttcgccgtccactttgtctaccgttactatgcggcttgcaaacccgacaacctccgttacttccaaggatgctactttgtcgcatgggtattcggagcaatggcggtggcggcgagctgggggttcgcagcgtttattctgtacccggagaccgagaggaccaggacggcgttgatacacgtcatacaaacatcctatgagctggatcccgagtgggtgggaaatgttccatatagctattggcgcacagaaaacggagtggaatacctgaatcctcgcaacgtcatcgggatctttcaacacggcgtcatcatgatcctctccttcggaacagtcttctactgcggattcaacacttataagactttgaacggaagtctgggggtgtctgaaaaaacatccggagtcgacaaagaaatgcacacccaattgttcaaggccttggttctacagactatcatccctactacactaatgtacatcccgacaaccatgctctttgtcaccccattcgttggactcaacatcggctgttacggcaacatcactactgccaccgtccatttgtatcctggaattgacccagtcgttttgatctttataatccgagacttccggcaaacgattttaagaccattcagatgcttctaccgttcaaatagtgtcgaaaacactgccaccataaggcaataccagcagagcagctccaaaggatctagagaattcggtacctaa